European Patent Specification EP 3 529 375 B1, published November 12, 2025. Title: Amplification-integrated genetic material depletion of non-target organisms using differentially abundant k-mers. Applicant: Siemens Healthcare GmbH. The sequence listing filed with the application follows.

SEQUENCE LISTING (486 sequences)

SEQ ID NO: 1 - DNA, 6 bp, Artificial Sequence
  k-mer
  misc_feature (3)..(6): n is a, c, g, or t
cgnnnn

SEQ ID NO: 2 - DNA, 6 bp, Artificial Sequence
  k-mer
  misc_feature (1)..(1): n is a, c, g, or t
  misc_feature (4)..(6): n is a, c, g, or t
ncgnnn

SEQ ID NO: 3 - DNA, 6 bp, Artificial Sequence
  k-mer
  misc_feature (1)..(2): n is a, c, g, or t
  misc_feature (5)..(6): n is a, c, g, or t
nncgnn

SEQ ID NO: 4 - DNA, 6 bp, Artificial Sequence
  k-mer
  misc_feature (1)..(3): n is a, c, g, or t
  misc_feature (6)..(6): n is a, c, g, or t
nnncgn

SEQ ID NO: 5 - DNA, 6 bp, Artificial Sequence
  k-mer
  misc_feature (1)..(4): n is a, c, g, or t
nnnncg

SEQ ID NO: 6 - DNA, 6 bp, Artificial Sequence
  k-mer
  misc_feature (5)..(6): n is a, c, g, or t
cgcgnn

SEQ ID NO: 7 - DNA, 6 bp, Artificial Sequence
  k-mer
  misc_feature (3)..(3): n is a, c, g, or t
  misc_feature (6)..(6): n is a, c, g, or t
cgncgn

SEQ ID NO: 8 - DNA, 6 bp, Artificial Sequence
  k-mer
  misc_feature (3)..(4): n is a, c, g, or t
cgnncg

SEQ ID NO: 9 - DNA, 6 bp, Artificial Sequence
  k-mer
  misc_feature (1)..(1): n is a, c, g, or t
  misc_feature (6)..(6): n is a, c, g, or t
ncgcgn

SEQ ID NO: 10 - DNA, 6 bp, Artificial Sequence
  k-mer
  misc_feature (1)..(1): n is a, c, g, or t
  misc_feature (4)..(4): n is a, c, g, or t
ncgncg

SEQ ID NO: 11 - DNA, 6 bp, Artificial Sequence
  k-mer
  misc_feature (1)..(2): n is a, c, g, or t
nncgcg

SEQ ID NO: 12 - DNA, 6 bp, Artificial Sequence
  k-mer
cgcgcg

SEQ ID NO: 13 - DNA, 7 bp, Artificial Sequence
  k-mer
  misc_feature (3)..(7): n is a, c, g, or t
cgnnnnn

SEQ ID NO: 14 - DNA, 7 bp, Artificial Sequence
  k-mer
  misc_feature (1)..(1): n is a, c, g, or t
  misc_feature (4)..(7): n is a, c, g, or t
ncgnnnn

SEQ ID NO: 15 - DNA, 7 bp, Artificial Sequence
  k-mer
  misc_feature (1)..(2): n is a, c, g, or t
  misc_feature (5)..(7): n is a, c, g, or t
nncgnnn

SEQ ID NO: 16 - DNA, 7 bp, Artificial Sequence
  k-mer
  misc_feature (1)..(3): n is a, c, g, or t
  misc_feature (6)..(7): n is a, c, g, or t
nnncgnn

SEQ ID NO: 17 - DNA, 7 bp, Artificial Sequence
  k-mer
  misc_feature (1)..(4): n is a, c, g, or t
  misc_feature (7)..(7): n is a, c, g, or t
nnnncgn

SEQ ID NO: 18 - DNA, 7 bp, Artificial Sequence
  k-mer
  misc_feature (1)..(5): n is a, c, g, or t
nnnnncg

SEQ ID NO: 19 - DNA, 7 bp, Artificial Sequence
  k-mer
  misc_feature (5)..(7): n is a, c, g, or t
cgcgnnn

SEQ ID NO: 20 - DNA, 7 bp, Artificial Sequence
  k-mer
  misc_feature (3)..(3): n is a, c, g, or t
  misc_feature (6)..(7): n is a, c, g, or t
cgncgnn

SEQ ID NO: 21 - DNA, 7 bp, Artificial Sequence
  k-mer
  misc_feature (3)..(4): n is a, c, g, or t
  misc_feature (7)..(7): n is a, c, g, or t
cgnncgn

SEQ ID NO: 22 - DNA, 7 bp, Artificial Sequence
  k-mer
  misc_feature (3)..(5): n is a, c, g, or t
cgnnncg

SEQ ID NO: 23 - DNA, 7 bp, Artificial Sequence
  k-mer
  misc_feature (1)..(1): n is a, c, g, or t
  misc_feature (6)..(7): n is a, c, g, or t
ncgcgnn

SEQ ID NO: 24 - DNA, 7 bp, Artificial Sequence
  k-mer
  misc_feature (1)..(1): n is a, c, g, or t
  misc_feature (4)..(4): n is a, c, g, or t
  misc_feature (7)..(7): n is a, c, g, or t
ncgncgn

SEQ ID NO: 25 - DNA, 7 bp, Artificial Sequence
  k-mer
  misc_feature (1)..(1): n is a, c, g, or t
  misc_feature (4)..(5): n is a, c, g, or t
ncgnncg

SEQ ID NO: 26 - DNA, 7 bp, Artificial Sequence
  k-mer
  misc_feature (1)..(2): n is a, c, g, or t
  misc_feature (7)..(7): n is a, c, g, or t
nncgcgn

SEQ ID NO: 27 - DNA, 7 bp, Artificial Sequence
  k-mer
  misc_feature (1)..(2): n is a, c, g, or t
  misc_feature (5)..(5): n is a, c, g, or t
nncgncg

SEQ ID NO: 28 - DNA, 7 bp, Artificial Sequence
  k-mer
  misc_feature (1)..(3): n is a, c, g, or t
nnncgcg

SEQ ID NO: 29 - DNA, 7 bp, Artificial Sequence
  k-mer
  misc_feature (7)..(7): n is a, c, g, or t
cgcgcgn

SEQ ID NO: 30 - DNA, 7 bp, Artificial Sequence
  k-mer
  misc_feature (5)..(5): n is a, c, g, or t
cgcgncg

SEQ ID NO: 31 - DNA, 7 bp, Artificial Sequence
  k-mer
  misc_feature (3)..(3): n is a, c, g, or t
cgncgcg

SEQ ID NO: 32 - DNA, 7 bp, Artificial Sequence
  k-mer
  misc_feature (1)..(1): n is a, c, g, or t
ncgcgcg

SEQ ID NO: 33 - DNA, 8 bp, Artificial Sequence
  k-mer
  misc_feature (3)..(8): n is a, c, g, or t
cgnnnnnn

SEQ ID NO: 34 - DNA, 8 bp, Artificial Sequence
  k-mer
  misc_feature (1)..(1): n is a, c, g, or t
  misc_feature (4)..(8): n is a, c, g, or t
ncgnnnnn

SEQ ID NO: 35 - DNA, 8 bp, Artificial Sequence
  k-mer
  misc_feature (1)..(2): n is a, c, g, or t
  misc_feature (5)..(8): n is a, c, g, or t
nncgnnnn

SEQ ID NO: 36 - DNA, 8 bp, Artificial Sequence
  k-mer
  misc_feature (1)..(3): n is a, c, g, or t
  misc_feature (6)..(8): n is a, c, g, or t
nnncgnnn

SEQ ID NO: 37 - DNA, 8 bp, Artificial Sequence
  k-mer
  misc_feature (1)..(4): n is a, c, g, or t
  misc_feature (7)..(8): n is a, c, g, or t
nnnncgnn

SEQ ID NO: 38 - DNA, 8 bp, Artificial Sequence
  k-mer
  misc_feature (1)..(5): n is a, c, g, or t
  misc_feature (8)..(8): n is a, c, g, or t
nnnnncgn

SEQ ID NO: 39 - DNA, 8 bp, Artificial Sequence
  k-mer
  misc_feature (1)..(6): n is a, c, g, or t
nnnnnncg

SEQ ID NO: 40 - DNA, 8 bp, Artificial Sequence
  k-mer
  misc_feature (5)..(8): n is a, c, g, or t
cgcgnnnn

SEQ ID NO: 41 - DNA, 8 bp, Artificial Sequence
  k-mer
  misc_feature (3)..(3): n is a, c, g, or t
  misc_feature (6)..(8): n is a, c, g, or t
cgncgnnn

SEQ ID NO: 42 - DNA, 8 bp, Artificial Sequence
  k-mer
  misc_feature (3)..(4): n is a, c, g, or t
  misc_feature (7)..(8): n is a, c, g, or t
cgnncgnn

SEQ ID NO: 43 - DNA, 8 bp, Artificial Sequence
  k-mer
  misc_feature (3)..(5): n is a, c, g, or t
  misc_feature (8)..(8): n is a, c, g, or t
cgnnncgn

SEQ ID NO: 44 - DNA, 8 bp, Artificial Sequence
  k-mer
  misc_feature (3)..(6): n is a, c, g, or t
cgnnnncg

SEQ ID NO: 45 - DNA, 8 bp, Artificial Sequence
  k-mer
  misc_feature (1)..(1): n is a, c, g, or t
  misc_feature (6)..(8): n is a, c, g, or t
ncgcgnnn

SEQ ID NO: 46 - DNA, 8 bp, Artificial Sequence
  k-mer
  misc_feature (1)..(1): n is a, c, g, or t
  misc_feature (4)..(4): n is a, c, g, or t
  misc_feature (7)..(8): n is a, c, g, or t
ncgncgnn

SEQ ID NO: 47 - DNA, 8 bp, Artificial Sequence
  k-mer
  misc_feature (1)..(1): n is a, c, g, or t
  misc_feature (4)..(5): n is a, c, g, or t
  misc_feature (8)..(8): n is a, c, g, or t
ncgnncgn

SEQ ID NO: 48 - DNA, 8 bp, Artificial Sequence
  k-mer
  misc_feature (1)..(1): n is a, c, g, or t
  misc_feature (4)..(6): n is a, c, g, or t
ncgnnncg

SEQ ID NO: 49 - DNA, 8 bp, Artificial Sequence
  k-mer
  misc_feature (1)..(2): n is a, c, g, or t
  misc_feature (7)..(8): n is a, c, g, or t
nncgcgnn

SEQ ID NO: 50 - DNA, 8 bp, Artificial Sequence
  k-mer
  misc_feature (1)..(2): n is a, c, g, or t
  misc_feature (5)..(5): n is a, c, g, or t
  misc_feature (8)..(8): n is a, c, g, or t
nncgncgn

SEQ ID NO: 51 - DNA, 8 bp, Artificial Sequence
  k-mer
  misc_feature (1)..(2): n is a, c, g, or t
  misc_feature (5)..(6): n is a, c, g, or t
nncgnncg

SEQ ID NO: 52 - DNA, 8 bp, Artificial Sequence
  k-mer
  misc_feature (1)..(3): n is a, c, g, or t
  misc_feature (8)..(8): n is a, c, g, or t
nnncgcgn

SEQ ID NO: 53 - DNA, 8 bp, Artificial Sequence
  k-mer
  misc_feature (1)..(3): n is a, c, g, or t
  misc_feature (6)..(6): n is a, c, g, or t
nnncgncg

SEQ ID NO: 54 - DNA, 8 bp, Artificial Sequence
  k-mer
  misc_feature (1)..(4): n is a, c, g, or t
nnnncgcg

SEQ ID NO: 55 - DNA, 8 bp, Artificial Sequence
  k-mer
  misc_feature (7)..(8): n is a, c, g, or t
cgcgcgnn

SEQ ID NO: 56 - DNA, 8 bp, Artificial Sequence
  k-mer
  misc_feature (5)..(5): n is a, c, g, or t
  misc_feature (8)..(8): n is a, c, g, or t
cgcgncgn

SEQ ID NO: 57 - DNA, 8 bp, Artificial Sequence
  k-mer
  misc_feature (5)..(6): n is a, c, g, or t
cgcgnncg

SEQ ID NO: 58 - DNA, 8 bp, Artificial Sequence
  k-mer
  misc_feature (3)..(3): n is a, c, g, or t
  misc_feature (8)..(8): n is a, c, g, or t
cgncgcgn

SEQ ID NO: 59 - DNA, 8 bp, Artificial Sequence
  k-mer
  misc_feature (3)..(3): n is a, c, g, or t
  misc_feature (6)..(6): n is a, c, g, or t
cgncgncg

SEQ ID NO: 60 - DNA, 8 bp, Artificial Sequence
  k-mer
  misc_feature (3)..(4): n is a, c, g, or t
cgnncgcg

SEQ ID NO: 61 - DNA, 8 bp, Artificial Sequence
  k-mer
  misc_feature (1)..(1): n is a, c, g, or t
  misc_feature (8)..(8): n is a, c, g, or t
ncgcgcgn

SEQ ID NO: 62 - DNA, 8 bp, Artificial Sequence
  k-mer
  misc_feature (1)..(1): n is a, c, g, or t
  misc_feature (6)..(6): n is a, c, g, or t
ncgcgncg

SEQ ID NO: 63 - DNA, 8 bp, Artificial Sequence
  k-mer
  misc_feature (1)..(1): n is a, c, g, or t
  misc_feature (4)..(4): n is a, c, g, or t
ncgncgcg

SEQ ID NO: 64 - DNA, 8 bp, Artificial Sequence
  k-mer
  misc_feature (1)..(2): n is a, c, g, or t
nncgcgcg

SEQ ID NO: 65 - DNA, 8 bp, Artificial Sequence
  k-mer
cgcgcgcg

SEQ ID NO: 66 - DNA, 6 bp, Artificial Sequence
  k-mer
  misc_feature (1)..(2): n is a, c, g, or t
nngcgc

SEQ ID NO: 67 - DNA, 6 bp, Artificial Sequence
  k-mer
  misc_feature (1)..(2): n is a, c, g, or t
nncggc

SEQ ID NO: 68 - DNA, 6 bp, Artificial Sequence
  k-mer
  misc_feature (1)..(1): n is a, c, g, or t
  misc_feature (6)..(6): n is a, c, g, or t
ngcgcn

SEQ ID NO: 69 - DNA, 6 bp, Artificial Sequence
  k-mer
  misc_feature (1)..(1): n is a, c, g, or t
  misc_feature (4)..(4): n is a, c, g, or t
ngcngc

SEQ ID NO: 70 - DNA, 6 bp, Artificial Sequence
  k-mer
  misc_feature (5)..(6): n is a, c, g, or t
gccgnn

SEQ ID NO: 71 - DNA, 6 bp, Artificial Sequence
  k-mer
  misc_feature (5)..(6): n is a, c, g, or t
gcgcnn

SEQ ID NO: 72 - DNA, 6 bp, Artificial Sequence
  k-mer
  misc_feature (3)..(4): n is a, c, g, or t
cgnngc

SEQ ID NO: 73 - DNA, 6 bp, Artificial Sequence
  k-mer
  misc_feature (1)..(1): n is a, c, g, or t
  misc_feature (6)..(6): n is a, c, g, or t
ncggcn

SEQ ID NO: 74 - DNA, 6 bp, Artificial Sequence
  k-mer
  misc_feature (5)..(6): n is a, c, g, or t
cggcnn

SEQ ID NO: 75 - DNA, 6 bp, Artificial Sequence
  k-mer
  misc_feature (1)..(2): n is a, c, g, or t
nngccg

SEQ ID NO: 76 - DNA, 6 bp, Artificial Sequence
  k-mer
  misc_feature (1)..(1): n is a, c, g, or t
  misc_feature (6)..(6): n is a, c, g, or t
ngccgn

SEQ ID NO: 77 - DNA, 6 bp, Artificial Sequence
  k-mer
  misc_feature (1)..(1): n is a, c, g, or t
  misc_feature (4)..(4): n is a, c, g, or t
ngcncg

SEQ ID NO: 78 - DNA, 6 bp, Artificial Sequence
  k-mer
  misc_feature (3)..(3): n is a, c, g, or t
  misc_feature (6)..(6): n is a, c, g, or t
gcncgn

SEQ ID NO: 79 - DNA, 6 bp, Artificial Sequence
  k-mer
  misc_feature (1)..(1): n is a, c, g, or t
  misc_feature (4)..(4): n is a, c, g, or t
ncgngc

SEQ ID NO: 80 - DNA, 6 bp, Artificial Sequence
  k-mer
  misc_feature (3)..(3): n is a, c, g, or t
  misc_feature (6)..(6): n is a, c, g, or t
cgngcn

SEQ ID NO: 81 - DNA, 6 bp, Artificial Sequence
  k-mer
  misc_feature (3)..(3): n is a, c, g, or t
  misc_feature (6)..(6): n is a, c, g, or t
gcngcn

SEQ ID NO: 82 - DNA, 6 bp, Artificial Sequence
  k-mer
  misc_feature (3)..(4): n is a, c, g, or t
gcnngc

SEQ ID NO: 83 - DNA, 6 bp, Artificial Sequence
  k-mer
  misc_feature (3)..(4): n is a, c, g, or t
gcnncg

SEQ ID NO: 84 - DNA, 6 bp, Artificial Sequence
  k-mer
  misc_feature (6)..(6): n is a, c, g, or t
cgacgn

SEQ ID NO: 85 - DNA, 6 bp, Artificial Sequence
  k-mer
cgacgc

SEQ ID NO: 86 - DNA, 6 bp, Artificial Sequence
  k-mer
cggcgc

SEQ ID NO: 87 - DNA, 8 bp, Artificial Sequence
  k-mer
cgacgata

SEQ ID NO: 88 - DNA, 8 bp, Artificial Sequence
  k-mer
gcgcgtaa

SEQ ID NO: 89 - DNA, 8 bp, Artificial Sequence
  k-mer
attacgcg

SEQ ID NO: 90 - DNA, 8 bp, Artificial Sequence
  k-mer
cgtcgata

SEQ ID NO: 91 - DNA, 8 bp, Artificial Sequence
  k-mer
cgataacg

SEQ ID NO: 92 - DNA, 8 bp, Artificial Sequence
  k-mer
cgcgataa

SEQ ID NO: 93 - DNA, 8 bp, Artificial Sequence
  k-mer
cgataccg

SEQ ID NO: 94 - DNA, 8 bp, Artificial Sequence
  k-mer
cgccgata

SEQ ID NO: 95 - DNA, 8 bp, Artificial Sequence
  k-mer
tatcgcga

SEQ ID NO: 96 - DNA, 8 bp, Artificial Sequence
  k-mer
cgcgtaaa

SEQ ID NO: 97 - DNA, 8 bp, Artificial Sequence
  k-mer
atcgtcgc

SEQ ID NO: 98 - DNA, 8 bp, Artificial Sequence
  k-mer
cggcgata

SEQ ID NO: 99 - DNA, 8 bp, Artificial Sequence
  k-mer
cgatacgc

SEQ ID NO: 100 - DNA, 8 bp, Artificial Sequence
  k-mer
atcgcgat

SEQ ID NO: 101 - DNA, 8 bp, Artificial Sequence
  k-mer
cggtacgc

SEQ ID NO: 102 - DNA, 8 bp, Artificial Sequence
  k-mer
attgcgcg

SEQ ID NO: 103 - DNA, 8 bp, Artificial Sequence
  k-mer
aatcgacg

SEQ ID NO: 104 - DNA, 8 bp, Artificial Sequence
  k-mer
cgatagcg

SEQ ID NO: 105 - DNA, 8 bp, Artificial Sequence
  k-mer
cgttacgc

SEQ ID NO: 106 - DNA, 8 bp, Artificial Sequence
  k-mer
ataacgcg

SEQ ID NO: 107 - DNA, 8 bp, Artificial Sequence
  k-mer
cgcgatac

SEQ ID NO: 108 - DNA, 8 bp, Artificial Sequence
  k-mer
cgcgaata

SEQ ID NO: 109 - DNA, 8 bp, Artificial Sequence
  k-mer
tcgcgtaa

SEQ ID NO: 110 - DNA, 8 bp, Artificial Sequence
  k-mer
aacgcgat

SEQ ID NO: 111 - DNA, 8 bp, Artificial Sequence
  k-mer
atttcgcg

SEQ ID NO: 112 - DNA, 8 bp, Artificial Sequence
  k-mer
cgtatcga

SEQ ID NO: 113 - DNA, 8 bp, Artificial Sequence
  k-mer
atcgacga

SEQ ID NO: 114 - DNA, 8 bp, Artificial Sequence
  k-mer
cgtaccga

SEQ ID NO: 115 - DNA, 8 bp, Artificial Sequence
  k-mer
tcgcgaaa

SEQ ID NO: 116 - DNA, 8 bp, Artificial Sequence
  k-mer
atacgcgc

SEQ ID NO: 117 - DNA, 8 bp, Artificial Sequence
  k-mer
cgatatcg

SEQ ID NO: 118 - DNA, 8 bp, Artificial Sequence
  k-mer
cgtaaacg

SEQ ID NO: 119 - DNA, 8 bp, Artificial Sequence
  k-mer
cgacgatc

SEQ ID NO: 120 - DNA, 8 bp, Artificial Sequence
  k-mer
cgattacg

SEQ ID NO: 121 - DNA, 8 bp, Artificial Sequence
  k-mer
aatcgtcg

SEQ ID NO: 122 - DNA, 8 bp, Artificial Sequence
  k-mer
cgccgtta

SEQ ID NO: 123 - DNA, 8 bp, Artificial Sequence
  k-mer
atcgacgc

SEQ ID NO: 124 - DNA, 8 bp, Artificial Sequence
  k-mer
cggcgtaa

SEQ ID NO: 125 - DNA, 8 bp, Artificial Sequence
  k-mer
cgtatcgc

SEQ ID NO: 126 - DNA, 8 bp, Artificial Sequence
  k-mer
atcgcgaa

SEQ ID NO: 127 - DNA, 8 bp, Artificial Sequence
  k-mer
tacgacga

SEQ ID NO: 128 - DNA, 8 bp, Artificial Sequence
  k-mer
atatcgcg

SEQ ID NO: 129 - DNA, 8 bp, Artificial Sequence
  k-mer
acgcgata

SEQ ID NO: 130 - DNA, 8 bp, Artificial Sequence
  k-mer
gcgtcgta

SEQ ID NO: 131 - DNA, 8 bp, Artificial Sequence
  k-mer
cgattgcg

SEQ ID NO: 132 - DNA, 8 bp, Artificial Sequence
  k-mer
cggtaacg

SEQ ID NO: 133 - DNA, 8 bp, Artificial Sequence
  k-mer
attcgtcg

SEQ ID NO: 134 - DNA, 8 bp, Artificial Sequence
  k-mer
cgcgtcga

SEQ ID NO: 135 - DNA, 8 bp, Artificial Sequence
  k-mer
gcgcgata

SEQ ID NO: 136 - DNA, 8 bp, Artificial Sequence
  k-mer
cgcgatta

SEQ ID NO: 137 - DNA, 8 bp, Artificial Sequence
  k-mer
acgcgtaa

SEQ ID NO: 138 - DNA, 8 bp, Artificial Sequence
  k-mer
cgttacga

SEQ ID NO: 139 - DNA, 8 bp, Artificial Sequence
  k-mer
tacgcgca

SEQ ID NO: 140 - DNA, 8 bp, Artificial Sequence
  k-mer
cgcgtaac

SEQ ID NO: 141 - DNA, 8 bp, Artificial Sequence
  k-mer
cgtaccgc

SEQ ID NO: 142 - DNA, 8 bp, Artificial Sequence
  k-mer
atcgcgcg

SEQ ID NO: 143 - DNA, 8 bp, Artificial Sequence
  k-mer
cgtcgtaa

SEQ ID NO: 144 - DNA, 8 bp, Artificial Sequence
  k-mer
aatacgcg

SEQ ID NO: 145 - DNA, 8 bp, Artificial Sequence
  k-mer
atcggcga

SEQ ID NO: 146 - DNA, 8 bp, Artificial Sequence
  k-mer
cgcgaaaa

SEQ ID NO: 147 - DNA, 8 bp, Artificial Sequence
  k-mer
tacgcgaa

SEQ ID NO: 148 - DNA, 8 bp, Artificial Sequence
  k-mer
acgtatcg

SEQ ID NO: 149 - DNA, 8 bp, Artificial Sequence
  k-mer
gtacgcga

SEQ ID NO: 150 - DNA, 8 bp, Artificial Sequence
  k-mer
attcgcga

SEQ ID NO: 151 - DNA, 8 bp, Artificial Sequence
  k-mer
acgacgat

SEQ ID NO: 152 - DNA, 8 bp, Artificial Sequence
  k-mer
cgcgaacg

SEQ ID NO: 153 - DNA, 8 bp, Artificial Sequence
  k-mer
cgcgacga

SEQ ID NO: 154 - DNA, 8 bp, Artificial Sequence
  k-mer
cgcgacaa

SEQ ID NO: 155 - DNA, 8 bp, Artificial Sequence
  k-mer
cgtaacga

SEQ ID NO: 156 - DNA, 8 bp, Artificial Sequence
  k-mer
attcgcgc

SEQ ID NO: 157 - DNA, 8 bp, Artificial Sequence
  k-mer
atcgtcga

SEQ ID NO: 158 - DNA, 8 bp, Artificial Sequence
  k-mer
atcgacgg

SEQ ID NO: 159 - DNA, 8 bp, Artificial Sequence
  k-mer
ccgcgata

SEQ ID NO: 160 - DNA, 8 bp, Artificial Sequence
  k-mer
acgaatcg

SEQ ID NO: 161 - DNA, 8 bp, Artificial Sequence
  k-mer
acgacgcg

SEQ ID NO: 162 - DNA, 8 bp, Artificial Sequence
  k-mer
cgaatacg

SEQ ID NO: 163 - DNA, 8 bp, Artificial Sequence
  k-mer
agcgcgta

SEQ ID NO: 164 - DNA, 8 bp, Artificial Sequence
  k-mer
atcgttcg

SEQ ID NO: 165 - DNA, 8 bp, Artificial Sequence
  k-mer
gcgcgtta

SEQ ID NO: 166 - DNA, 8 bp, Artificial Sequence
  k-mer
atgcgacg

SEQ ID NO: 167 - DNA, 8 bp, Artificial Sequence
  k-mer
gtcgcgta

SEQ ID NO: 168 - DNA, 8 bp, Artificial Sequence
  k-mer
acgcgcaa

SEQ ID NO: 169 - DNA, 8 bp, Artificial Sequence
  k-mer
acgatacg

SEQ ID NO: 170 - DNA, 8 bp, Artificial Sequence
  k-mer
tcgcgcaa

SEQ ID NO: 171 - DNA, 8 bp, Artificial Sequence
  k-mer
aatgcgcg

SEQ ID NO: 172 - DNA, 8 bp, Artificial Sequence
  k-mer
cgcggtaa

SEQ ID NO: 173 - DNA, 8 bp, Artificial Sequence
  k-mer
cggtacga

SEQ ID NO: 174 - DNA, 8 bp, Artificial Sequence
  k-mer
taccgcga

SEQ ID NO: 175 - DNA, 8 bp, Artificial Sequence
  k-mer
aacgcgta

SEQ ID NO: 176 - DNA, 8 bp, Artificial Sequence
  k-mer
atacgccg

SEQ ID NO: 177 - DNA, 8 bp, Artificial Sequence
  k-mer
cgacggta

SEQ ID NO: 178 - DNA, 8 bp, Artificial Sequence
  k-mer
ccgatacg

SEQ ID NO: 179 - DNA, 8 bp, Artificial Sequence
  k-mer
gcgcgaaa

SEQ ID NO: 180 - DNA, 8 bp, Artificial Sequence
  k-mer
cgtcgtta

SEQ ID NO: 181 - DNA, 8 bp, Artificial Sequence
  k-mer
tgcgcgaa

SEQ ID NO: 182 - DNA, 8 bp, Artificial Sequence
  k-mer
cgtcaacg

SEQ ID NO: 183 - DNA, 8 bp, Artificial Sequence
  k-mer
tcgacgaa

SEQ ID NO: 184 - DNA, 8 bp, Artificial Sequence
  k-mer
cgcgcata

SEQ ID NO: 185 - DNA, 8 bp, Artificial Sequence
  k-mer
cgtcgtac

SEQ ID NO: 186 - DNA, 8 bp, Artificial Sequence
  k-mer
cgttgcga

SEQ ID NO: 187 - DNA, 6 bp, Artificial Sequence
  k-mer
cgtcga

SEQ ID NO: 188 - DNA, 6 bp, Artificial Sequence
  k-mer
cgacga

SEQ ID NO: 189 - DNA, 6 bp, Artificial Sequence
  k-mer
cgacgc

SEQ ID NO: 190 - DNA, 6 bp, Artificial Sequence
  k-mer
cgatcg

SEQ ID NO: 191 - DNA, 6 bp, Artificial Sequence
  k-mer
cgtcgc

SEQ ID NO: 192 - DNA, 6 bp, Artificial Sequence
  k-mer
acgacg

SEQ ID NO: 193 - DNA, 6 bp, Artificial Sequence
  k-mer
cgcgac

SEQ ID NO: 194 - DNA, 6 bp, Artificial Sequence
  k-mer
cgaccg

SEQ ID NO: 195 - DNA, 6 bp, Artificial Sequence
  k-mer
cgccga

SEQ ID NO: 196 - DNA, 6 bp, Artificial Sequence
  k-mer
acgtcg

SEQ ID NO: 197 - DNA, 6 bp, Artificial Sequence
  k-mer
tcgcga

SEQ ID NO: 198 - DNA, 6 bp, Artificial Sequence
  k-mer
acgcgc

SEQ ID NO: 199 - DNA, 6 bp, Artificial Sequence
  k-mer
cgcgta

SEQ ID NO: 200 - DNA, 6 bp, Artificial Sequence
  k-mer
gtcgac

SEQ ID NO: 201 - DNA, 6 bp, Artificial Sequence
  k-mer
acgcga

SEQ ID NO: 202 - DNA, 6 bp, Artificial Sequence
  k-mer
cgcgaa

SEQ ID NO: 203 - DNA, 6 bp, Artificial Sequence
  k-mer
aacgcg

SEQ ID NO: 204 - DNA, 6 bp, Artificial Sequence
  k-mer
cgtacg

SEQ ID NO: 205 - DNA, 6 bp, Artificial Sequence
  k-mer
gacgac

SEQ ID NO: 206 - DNA, 6 bp, Artificial Sequence
  k-mer
acgcgt

SEQ ID NO: 207 - DNA, 6 bp, Artificial Sequence
  k-mer
cgaacg

SEQ ID NO: 208 - DNA, 6 bp, Artificial Sequence
  k-mer
atcgac

SEQ ID NO: 209 - DNA, 6 bp, Artificial Sequence
  k-mer
atcgcg

SEQ ID NO: 210 - DNA, 6 bp, Artificial Sequence
  k-mer
gcgcaa

SEQ ID NO: 211 - DNA, 6 bp, Artificial Sequence
  k-mer
cgccaa

SEQ ID NO: 212 - DNA, 6 bp, Artificial Sequence
  k-mer
cgacaa

SEQ ID NO: 213 - DNA, 6 bp, Artificial Sequence
  k-mer
atgcgc

SEQ ID NO: 214 - DNA, 6 bp, Artificial Sequence
  k-mer
gtcgca

SEQ ID NO: 215 - DNA, 6 bp, Artificial Sequence
  k-mer
cgatgc

SEQ ID NO: 216 - DNA, 6 bp, Artificial Sequence
  k-mer
gcgtac

SEQ ID NO: 217 - DNA, 6 bp, Artificial Sequence
  k-mer
acgacc

SEQ ID NO: 218 - DNA, 6 bp, Artificial Sequence
  k-mer
gcggta

SEQ ID NO: 219 - DNA, 6 bp, Artificial Sequence
  k-mer
caacgc

SEQ ID NO: 220 - DNA, 6 bp, Artificial Sequence
  k-mer
tgcgca

SEQ ID NO: 221 - DNA, 6 bp, Artificial Sequence
  k-mer
atcgtc

SEQ ID NO: 222 - DNA, 6 bp, Artificial Sequence
  k-mer
cgcaac

SEQ ID NO: 223 - DNA, 6 bp, Artificial Sequence
  k-mer
catcgc

SEQ ID NO: 224 - DNA, 6 bp, Artificial Sequence
  k-mer
cgatac

SEQ ID NO: 225 - DNA, 6 bp, Artificial Sequence
  k-mer
cgcatc

SEQ ID NO: 226 - DNA, 6 bp, Artificial Sequence
  k-mer
tcgaca

SEQ ID NO: 227 - DNA, 6 bp, Artificial Sequence
  k-mer
gcgata

SEQ ID NO: 228 - DNA, 6 bp, Artificial Sequence
  k-mer
agcgac

SEQ ID NO: 229 - DNA, 6 bp, Artificial Sequence
  k-mer
cgataa

SEQ ID NO: 230 - DNA, 6 bp, Artificial Sequence
  k-mer
cgttgc

SEQ ID NO: 231 - DNA, 6 bp, Artificial Sequence
  k-mer
gcgtca

SEQ ID NO: 232 - DNA, 6 bp, Artificial Sequence
  k-mer
gcgaac

SEQ ID NO: 233 - DNA, 6 bp, Artificial Sequence
  k-mer
aacgcc

SEQ ID NO: 234 - DNA, 6 bp, Artificial Sequence
  k-mer
atgtcg

SEQ ID NO: 235 - DNA, 6 bp, Artificial Sequence
  k-mer
cggtac

SEQ ID NO: 236 - DNA, 6 bp, Artificial Sequence
  k-mer
caatcg

SEQ ID NO: 237 - DNA, 6 bp, Artificial Sequence
  k-mer
tatcga

SEQ ID NO: 238 - DNA, 6 bp, Artificial Sequence
  k-mer
cgcaaa

SEQ ID NO: 239 - DNA, 6 bp, Artificial Sequence
  k-mer
accgat

SEQ ID NO: 240 - DNA, 6 bp, Artificial Sequence
  k-mer
aagcgc

SEQ ID NO: 241 - DNA, 6 bp, Artificial Sequence
  k-mer
gcgcta

SEQ ID NO: 242 - DNA, 6 bp, Artificial Sequence
  k-mer
gtcgta

SEQ ID NO: 243 - DNA, 6 bp, Artificial Sequence
  k-mer
ccgata

SEQ ID NO: 244 - DNA, 6 bp, Artificial Sequence
  k-mer
gcgtaa

SEQ ID NO: 245 - DNA, 6 bp, Artificial Sequence
  k-mer
catcga

SEQ ID NO: 246 - DNA, 6 bp, Artificial Sequence
  k-mer
ggcgta

SEQ ID NO: 247 - DNA, 6 bp, Artificial Sequence
  k-mer
attcgc

SEQ ID NO: 248 - DNA, 6 bp, Artificial Sequence
  k-mer
atcgat

SEQ ID NO: 249 - DNA, 6 bp, Artificial Sequence
  k-mer
cgtcaa

SEQ ID NO: 250 - DNA, 6 bp, Artificial Sequence
  k-mer
aacgac

SEQ ID NO: 251 - DNA, 6 bp, Artificial Sequence
  k-mer
atatcg

SEQ ID NO: 252 - DNA, 6 bp, Artificial Sequence
  k-mer
acgaca

SEQ ID NO: 253 - DNA, 6 bp, Artificial Sequence
  k-mer
cgatga

SEQ ID NO: 254 - DNA, 6 bp, Artificial Sequence
  k-mer
ataccg

SEQ ID NO: 255 - DNA, 6 bp, Artificial Sequence
  k-mer
cgctac

SEQ ID NO: 256 - DNA, 6 bp, Artificial Sequence
  k-mer
aatgcg

SEQ ID NO: 257 - DNA, 6 bp, Artificial Sequence
  k-mer
tcgcaa

SEQ ID NO: 258 - DNA, 6 bp, Artificial Sequence
  k-mer
gtcgaa

SEQ ID NO: 259 - DNA, 6 bp, Artificial Sequence
  k-mer
caacga

SEQ ID NO: 260 - DNA, 6 bp, Artificial Sequence
  k-mer
attgcg

SEQ ID NO: 261 - DNA, 6 bp, Artificial Sequence
  k-mer
cgttga

SEQ ID NO: 262 - DNA, 6 bp, Artificial Sequence
  k-mer
cgatca

SEQ ID NO: 263 - DNA, 6 bp, Artificial Sequence
  k-mer
tcgtca

SEQ ID NO: 264 - DNA, 6 bp, Artificial Sequence
  k-mer
gcgaaa

SEQ ID NO: 265 - DNA, 6 bp, Artificial Sequence
  k-mer
atacgc

SEQ ID NO: 266 - DNA, 6 bp, Artificial Sequence
  k-mer
taccga

SEQ ID NO: 267 - DNA, 6 bp, Artificial Sequence
  k-mer
atgcga

SEQ ID NO: 268 - DNA, 6 bp, Artificial Sequence
  k-mer
cgtacc

SEQ ID NO: 269 - DNA, 6 bp, Artificial Sequence
  k-mer
aaagcg

SEQ ID NO: 270 - DNA, 6 bp, Artificial Sequence
  k-mer
atgacg

SEQ ID NO: 271 - DNA, 6 bp, Artificial Sequence
  k-mer
gtacga

SEQ ID NO: 272 - DNA, 6 bp, Artificial Sequence
  k-mer
cgaaaa

SEQ ID NO: 273 - DNA, 6 bp, Artificial Sequence
  k-mer
acgata

SEQ ID NO: 274 - DNA, 6 bp, Artificial Sequence
  k-mer
cggata

SEQ ID NO: 275 - DNA, 6 bp, Artificial Sequence
  k-mer
cggtta

SEQ ID NO: 276 - DNA, 6 bp, Artificial Sequence
  k-mer
agtcga

SEQ ID NO: 277 - DNA, 6 bp, Artificial Sequence
  k-mer
cgacta

SEQ ID NO: 278 - DNA, 6 bp, Artificial Sequence
  k-mer
cgcata

SEQ ID NO: 279 - DNA, 6 bp, Artificial Sequence
  k-mer
acgcaa

SEQ ID NO: 280 - DNA, 6 bp, Artificial Sequence
  k-mer
atagcg

SEQ ID NO: 281 - DNA, 6 bp, Artificial Sequence
  k-mer
gacgaa

SEQ ID NO: 282 - DNA, 6 bp, Artificial Sequence
  k-mer
aacggt

SEQ ID NO: 283 - DNA, 6 bp, Artificial Sequence
  k-mer
acaacg

SEQ ID NO: 284 - DNA, 6 bp, Artificial Sequence
  k-mer
cgatag

SEQ ID NO: 285 - DNA, 6 bp, Artificial Sequence
  k-mer
acatcg

SEQ ID NO: 286 - DNA, 6 bp, Artificial Sequence
  k-mer
acgatg

SEQ ID NO: 287 - DNA, 7 bp, Artificial Sequence
  k-mer
cgtcgac

SEQ ID NO: 288 - DNA, 7 bp, Artificial Sequence
  k-mer
cgacgac

SEQ ID NO: 289 - DNA, 7 bp, Artificial Sequence
  k-mer
cgcgacg

SEQ ID NO: 290 - DNA, 7 bp, Artificial Sequence
  k-mer
cgacgcg

SEQ ID NO: 291 - DNA, 7 bp, Artificial Sequence
  k-mer
gcgtcga

SEQ ID NO: 292 - DNA, 7 bp, Artificial Sequence
  k-mer
tcgacga

SEQ ID NO: 293 - DNA, 7 bp, Artificial Sequence
  k-mer
cgcgcga

SEQ ID NO: 294 - DNA, 7 bp, Artificial Sequence
  k-mer
cgtcgtc

SEQ ID NO: 295 - DNA, 7 bp, Artificial Sequence
  k-mer
gcgacga

SEQ ID NO: 296 - DNA, 7 bp, Artificial Sequence
  k-mer
ccgtcga

SEQ ID NO: 297 - DNA, 7 bp, Artificial Sequence
  k-mer
atcgtcg

SEQ ID NO: 298 - DNA, 7 bp, Artificial Sequence
  k-mer
atcgacg

SEQ ID NO: 299 - DNA, 7 bp, Artificial Sequence
  k-mer
cggtcga

SEQ ID NO: 300 - DNA, 7 bp, Artificial Sequence
  k-mer
cgtcgag

SEQ ID NO: 301 - DNA, 7 bp, Artificial Sequence
  k-mer
cgcgcaa

SEQ ID NO: 302 - DNA, 7 bp, Artificial Sequence
  k-mer
atcggcg

SEQ ID NO: 303 - DNA, 7 bp, Artificial Sequence
  k-mer
acgacga

SEQ ID NO: 304 - DNA, 7 bp, Artificial Sequence
  k-mer
cgatcga

SEQ ID NO: 305 - DNA, 7 bp, Artificial Sequence
  k-mer
ccgacga

SEQ ID NO: 306 - DNA, 7 bp, Artificial Sequence
  k-mer
cgatcgc

SEQ ID NO: 307 - DNA, 7 bp, Artificial Sequence
  k-mer
atcgccg

SEQ ID NO: 308 - DNA, 7 bp, Artificial Sequence
  k-mer
cgaccga

SEQ ID NO: 309 - DNA, 7 bp, Artificial Sequence
  k-mer
acgtcga

SEQ ID NO: 310 - DNA, 7 bp, Artificial Sequence
  k-mer
cgacgtc

SEQ ID NO: 311 - DNA, 7 bp, Artificial Sequence
  k-mer
acgacgc

SEQ ID NO: 312 - DNA, 7 bp, Artificial Sequence
  k-mer
cggtacg

SEQ ID NO: 313 - DNA, 7 bp, Artificial Sequence
  k-mer
accgacg

SEQ ID NO: 314 - DNA, 7 bp, Artificial Sequence
  k-mer
cgcgata

SEQ ID NO: 315 - DNA, 7 bp, Artificial Sequence
  k-mer
ccgatcg

SEQ ID NO: 316 - DNA, 7 bp, Artificial Sequence
  k-mer
accgtcg

SEQ ID NO: 317 - DNA, 7 bp, Artificial Sequence
  k-mer
tcgcgca

SEQ ID NO: 318 - DNA, 7 bp, Artificial Sequence
  k-mer
gcgcgta

SEQ ID NO: 319 - DNA, 7 bp, Artificial Sequence
  k-mer
cgacgag

SEQ ID NO: 320 - DNA, 7 bp, Artificial Sequence
  k-mer
acgcgac

SEQ ID NO: 321 - DNA, 7 bp, Artificial Sequence
  k-mer
cgaccgc

SEQ ID NO: 322 - DNA, 7 bp, Artificial Sequence
  k-mer
cgcgaca

SEQ ID NO: 323 - DNA, 7 bp, Artificial Sequence
  k-mer
tcgccga

SEQ ID NO: 324 - DNA, 7 bp, Artificial Sequence
  k-mer
gtcgcga

SEQ ID NO: 325 - DNA, 7 bp, Artificial Sequence
  k-mer
cgcgaaa

SEQ ID NO: 326 - DNA, 7 bp, Artificial Sequence
  k-mer
cggcgta

SEQ ID NO: 327 - DNA, 7 bp, Artificial Sequence
  k-mer
gacgcgc

SEQ ID NO: 328 - DNA, 7 bp, Artificial Sequence
  k-mer
gcgccga

SEQ ID NO: 329 - DNA, 7 bp, Artificial Sequence
  k-mer
cgcaacg

SEQ ID NO: 330 - DNA, 7 bp, Artificial Sequence
  k-mer
cgcacga

SEQ ID NO: 331 - DNA, 7 bp, Artificial Sequence
  k-mer
acgaccg

SEQ ID NO: 332 - DNA, 7 bp, Artificial Sequence
  k-mer
cgcgtaa

SEQ ID NO: 333 - DNA, 7 bp, Artificial Sequence
  k-mer
cgatacg

SEQ ID NO: 334 - DNA, 7 bp, Artificial Sequence
  k-mer
acggtcg

SEQ ID NO: 335 - DNA, 7 bp, Artificial Sequence
  k-mer
atgcgcg

SEQ ID NO: 336 - DNA, 7 bp, Artificial Sequence
  k-mer
cgtcgca

SEQ ID NO: 337 - DNA, 7 bp, Artificial Sequence
  k-mer
acgacgg

SEQ ID NO: 338 - DNA, 7 bp, Artificial Sequence
  k-mer
acgtcgc

SEQ ID NO: 339 - DNA, 7 bp, Artificial Sequence
  k-mer
acgccga

SEQ ID NO: 340 - DNA, 7 bp, Artificial Sequence
  k-mer
acgatcg

SEQ ID NO: 341 - DNA, 7 bp, Artificial Sequence
  k-mer
acggcga

SEQ ID NO: 342 - DNA, 7 bp, Artificial Sequence
  k-mer
cgccgta

SEQ ID NO: 343 - DNA, 7 bp, Artificial Sequence
  k-mer
cgacgaa

SEQ ID NO: 344 - DNA, 7 bp, Artificial Sequence
  k-mer
atcgcga

SEQ ID NO: 345 - DNA, 7 bp, Artificial Sequence
  k-mer
cgacgca

SEQ ID NO: 346 - DNA, 7 bp, Artificial Sequence
  k-mer
gcgcgaa

SEQ ID NO: 347 - DNA, 7 bp, Artificial Sequence
  k-mer
cgaaccg

SEQ ID NO: 348 - DNA, 7 bp, Artificial Sequence
  k-mer
cgtcgta

SEQ ID NO: 349 - DNA, 7 bp, Artificial Sequence
  k-mer
cgacacg

SEQ ID NO: 350 - DNA, 7 bp, Artificial Sequence
  k-mer
agcgtcg

SEQ ID NO: 351 - DNA, 7 bp, Artificial Sequence
  k-mer
cgatgcg

SEQ ID NO: 352 - DNA, 7 bp, Artificial Sequence
  k-mer
cgctacg

SEQ ID NO: 353 - DNA, 7 bp, Artificial Sequence
  k-mer
cgccgaa

SEQ ID NO: 354 - DNA, 7 bp, Artificial Sequence
  k-mer
tacgcga

SEQ ID NO: 355 - DNA, 7 bp, Artificial Sequence
  k-mer
aacgcgc

SEQ ID NO: 356 - DNA, 7 bp, Artificial Sequence
  k-mer
attcgcg

SEQ ID NO: 357 - DNA, 7 bp, Artificial Sequence
  k-mer
cgcgtac

SEQ ID NO: 358 - DNA, 7 bp, Artificial Sequence
  k-mer
aacggcg

SEQ ID NO: 359 - DNA, 7 bp, Artificial Sequence
  k-mer
acgcgct

SEQ ID NO: 360 - DNA, 7 bp, Artificial Sequence
  k-mer
cacgacg

SEQ ID NO: 361 - DNA, 7 bp, Artificial Sequence
  k-mer
tcgcgaa

SEQ ID NO: 362 - DNA, 7 bp, Artificial Sequence
  k-mer
cgtcgaa

SEQ ID NO: 363 - DNA, 7 bp, Artificial Sequence
  k-mer
cgctcga

SEQ ID NO: 364 - DNA, 7 bp, Artificial Sequence
  k-mer
acgcgca

SEQ ID NO: 365 - DNA, 7 bp, Artificial Sequence
  k-mer
cgtacgc

SEQ ID NO: 366 - DNA, 7 bp, Artificial Sequence
  k-mer
catcgcg

SEQ ID NO: 367 - DNA, 7 bp, Artificial Sequence
  k-mer
cgtgcga

SEQ ID NO: 368 - DNA, 7 bp, Artificial Sequence
  k-mer
cgaatcg

SEQ ID NO: 369 - DNA, 7 bp, Artificial Sequence
  k-mer
cgactcg

SEQ ID NO: 370 - DNA, 7 bp, Artificial Sequence
  k-mer
aatcgcg

SEQ ID NO: 371 - DNA, 7 bp, Artificial Sequence
  k-mer
caacgcg

SEQ ID NO: 372 - DNA, 7 bp, Artificial Sequence
  k-mer
acgagcg

SEQ ID NO: 373 - DNA, 7 bp, Artificial Sequence
  k-mer
atacgcg

SEQ ID NO: 374 - DNA, 7 bp, Artificial Sequence
  k-mer
aacgacg

SEQ ID NO: 375 - DNA, 7 bp, Artificial Sequence
  k-mer
aagcgcg

SEQ ID NO: 376 - DNA, 7 bp, Artificial Sequence
  k-mer
acgccgt

SEQ ID NO: 377 - DNA, 7 bp, Artificial Sequence
  k-mer
cacgtcg

SEQ ID NO: 378 - DNA, 7 bp, Artificial Sequence
  k-mer
atcgcgg

SEQ ID NO: 379 - DNA, 7 bp, Artificial Sequence
  k-mer
aacgtcg

SEQ ID NO: 380 - DNA, 7 bp, Artificial Sequence
  k-mer
cgtaacg

SEQ ID NO: 381 - DNA, 7 bp, Artificial Sequence
  k-mer
cgcggta

SEQ ID NO: 382 - DNA, 7 bp, Artificial Sequence
  k-mer
agcgcga

SEQ ID NO: 383 - DNA, 7 bp, Artificial Sequence
  k-mer
gacgcga

SEQ ID NO: 384 - DNA, 7 bp, Artificial Sequence
  k-mer
acgacgt

SEQ ID NO: 385 - DNA, 7 bp, Artificial Sequence
  k-mer
cgacgta

SEQ ID NO: 386 - DNA, 7 bp, Artificial Sequence
  k-mer
acgcgtc

SEQ ID NO: 387 - DNA, 6 bp, Artificial Sequence
  k-mer
cgtcga

SEQ ID NO: 388 - DNA, 6 bp, Artificial Sequence
  k-mer
cgacga

SEQ ID NO: 389 - DNA, 6 bp, Artificial Sequence
  k-mer
cgatcg

SEQ ID NO: 390 - DNA, 6 bp, Artificial Sequence
  k-mer
cggcga

SEQ ID NO: 391 - DNA, 6 bp, Artificial Sequence
  k-mer
cgccga

SEQ ID NO: 392 - DNA, 6 bp, Artificial Sequence
  k-mer
cgcgaa

SEQ ID NO: 393 - DNA, 6 bp, Artificial Sequence
  k-mer
cgaccg

SEQ ID NO: 394 - DNA, 6 bp, Artificial Sequence
  k-mer
cgaacg

SEQ ID NO: 395 - DNA, 6 bp, Artificial Sequence
  k-mer
tcgcga

SEQ ID NO: 396 - DNA, 6 bp, Artificial Sequence
  k-mer
acgacg

SEQ ID NO: 397 - DNA, 6 bp, Artificial Sequence
  k-mer
ccgtcg

SEQ ID NO: 398 - DNA, 6 bp, Artificial Sequence
  k-mer
cgtcgc

SEQ ID NO: 399 - DNA, 6 bp, Artificial Sequence
  k-mer
cgacgc

SEQ ID NO: 400 - DNA, 6 bp, Artificial Sequence
  k-mer
acgccg

SEQ ID NO: 401 - DNA, 6 bp, Artificial Sequence
  k-mer
acggcg

SEQ ID NO: 402 - DNA, 6 bp, Artificial Sequence
  k-mer
cgcgac

SEQ ID NO: 403 - DNA, 6 bp, Artificial Sequence
  k-mer
ccgacg

SEQ ID NO: 404 - DNA, 6 bp, Artificial Sequence
  k-mer
cgcgta

SEQ ID NO: 405 - DNA, 6 bp, Artificial Sequence
  k-mer
acgtcg

SEQ ID NO: 406 - DNA, 6 bp, Artificial Sequence
  k-mer
aacgcg

SEQ ID NO: 407 - DNA, 6 bp, Artificial Sequence
  k-mer
ccgcga

SEQ ID NO: 408 - DNA, 6 bp, Artificial Sequence
  k-mer
acgcga

SEQ ID NO: 409 - DNA, 6 bp, Artificial Sequence
  k-mer
atcggc

SEQ ID NO: 410 - DNA, 6 bp, Artificial Sequence
  k-mer
cgagcg

SEQ ID NO: 411 - DNA, 6 bp, Artificial Sequence
  k-mer
ccggcg

SEQ ID NO: 412 - DNA, 6 bp, Artificial Sequence
  k-mer
cgtacg

SEQ ID NO: 413 - DNA, 6 bp, Artificial Sequence
  k-mer
atcgac

SEQ ID NO: 414 - DNA, 6 bp, Artificial Sequence
  k-mer
agcgcg

SEQ ID NO: 415 - DNA, 6 bp, Artificial Sequence
  k-mer
ccgccg

SEQ ID NO: 416 - DNA, 6 bp, Artificial Sequence
  k-mer
cgcgga

SEQ ID NO: 417 - DNA, 6 bp, Artificial Sequence
  k-mer
atcgcc

SEQ ID NO: 418 - DNA, 6 bp, Artificial Sequence
  k-mer
cggcgc

SEQ ID NO: 419 - DNA, 6 bp, Artificial Sequence
  k-mer
cgccgc

SEQ ID NO: 420 - DNA, 6 bp, Artificial Sequence
  k-mer
cgcgca

SEQ ID NO: 421 - DNA, 6 bp, Artificial Sequence
  k-mer
gcgaac

SEQ ID NO: 422 - DNA, 6 bp, Artificial Sequence
  k-mer
cgcgtc

SEQ ID NO: 423 - DNA, 6 bp, Artificial Sequence
  k-mer
cggcaa

SEQ ID NO: 424 - DNA, 6 bp, Artificial Sequence
  k-mer
ccgatc

SEQ ID NO: 425 - DNA, 6 bp, Artificial Sequence
  k-mer
cggacg

SEQ ID NO: 426 - DNA, 6 bp, Artificial Sequence
  k-mer
gccgac

SEQ ID NO: 427 - DNA, 6 bp, Artificial Sequence
  k-mer
cgcgag

SEQ ID NO: 428 - DNA, 6 bp, Artificial Sequence
  k-mer
acgcgg

SEQ ID NO: 429 - DNA, 6 bp, Artificial Sequence
  k-mer
gcggta

SEQ ID NO: 430 - DNA, 6 bp, Artificial Sequence
  k-mer
acgcgc

SEQ ID NO: 431 - DNA, 6 bp, Artificial Sequence
  k-mer
accggc

SEQ ID NO: 432 - DNA, 6 bp, Artificial Sequence
  k-mer
atcgcg

SEQ ID NO: 433 - DNA, 6 bp, Artificial Sequence
  k-mer
catcgg

SEQ ID NO: 434 - DNA, 6 bp, Artificial Sequence
  k-mer
cgatgc

SEQ ID NO: 435 - DNA, 6 bp, Artificial Sequence
  k-mer
atgccg

SEQ ID NO: 436 - DNA, 6 bp, Artificial Sequence
  k-mer
tcggca

SEQ ID NO: 437 - DNA, 6 bp, Artificial Sequence
  k-mer
gccgaa

SEQ ID NO: 438 - DNA, 6 bp, Artificial Sequence
  k-mer
cgcggc

SEQ ID NO: 439 - DNA, 6 bp, Artificial Sequence
  k-mer
cgatga

SEQ ID NO: 440 - DNA, 6 bp, Artificial Sequence
  k-mer
atcgtc

SEQ ID NO: 441 - DNA, 6 bp, Artificial Sequence
  k-mer
accgac

SEQ ID NO: 442 - DNA, 6 bp, Artificial Sequence
  k-mer
ccgaac

SEQ ID NO: 443 - DNA, 6 bp, Artificial Sequence
  k-mer
accgcc

SEQ ID NO: 444 - DNA, 6 bp, Artificial Sequence
  k-mer
gtcgaa

SEQ ID NO: 445 - DNA, 6 bp, Artificial Sequence
  k-mer
gcgacc

SEQ ID NO: 446 - DNA, 6 bp, Artificial Sequence
  k-mer
accgat

SEQ ID NO: 447 - DNA, 6 bp, Artificial Sequence
  k-mer
aacggc

SEQ ID NO: 448 - DNA, 6 bp, Artificial Sequence
  k-mer
catcga

SEQ ID NO: 449 - DNA, 6 bp, Artificial Sequence
  k-mer
catcgc

SEQ ID NO: 450 - DNA, 6 bp, Artificial Sequence
  k-mer
gccgta

SEQ ID NO: 451 - DNA, 6 bp, Artificial Sequence
  k-mer
gacgac

SEQ ID NO: 452 - DNA, 6 bp, Artificial Sequence
  k-mer
cgatac

SEQ ID NO: 453 - DNA, 6 bp, Artificial Sequence
  k-mer
cgccaa

SEQ ID NO: 454 - DNA, 6 bp, Artificial Sequence
  k-mer
gtcgac

SEQ ID NO: 455 - DNA, 6 bp, Artificial Sequence
  k-mer
ccgata

SEQ ID NO: 456 - DNA, 6 bp, Artificial Sequence
  k-mer
gaccgc

SEQ ID NO: 457 - DNA, 6 bp, Artificial Sequence
  k-mer
ggtcga

SEQ ID NO: 458 - DNA, 6 bp, Artificial Sequence
  k-mer
cgatca

SEQ ID NO: 459 - DNA, 6 bp, Artificial Sequence
  k-mer
cgcatc

SEQ ID NO: 460 - DNA, 6 bp, Artificial Sequence
  k-mer
cgacca

SEQ ID NO: 461 - DNA, 6 bp, Artificial Sequence
  k-mer
gacggc

SEQ ID NO: 462 - DNA, 6 bp, Artificial Sequence
  k-mer
accggt

SEQ ID NO: 463 - DNA, 6 bp, Artificial Sequence
  k-mer
atccgg

SEQ ID NO: 464 - DNA, 6 bp, Artificial Sequence
  k-mer
acgcgt

SEQ ID NO: 465 - DNA, 6 bp, Artificial Sequence
  k-mer
aacgcc

SEQ ID NO: 466 - DNA, 6 bp, Artificial Sequence
  k-mer
ccggta

SEQ ID NO: 467 - DNA, 6 bp, Artificial Sequence
  k-mer
cggtac

SEQ ID NO: 468 - DNA, 6 bp, Artificial Sequence
  k-mer
aaccgc

SEQ ID NO: 469 - DNA, 6 bp, Artificial Sequence
  k-mer
cgcacg

SEQ ID NO: 470 - DNA, 6 bp, Artificial Sequence
  k-mer
gcggca

SEQ ID NO: 471 - DNA, 6 bp, Artificial Sequence
  k-mer
caacgc

SEQ ID NO: 472 - DNA, 6 bp, Artificial Sequence
  k-mer
gcgcga

SEQ ID NO: 473 - DNA, 6 bp, Artificial Sequence
  k-mer
gcgtac

SEQ ID NO: 474 - DNA, 6 bp, Artificial Sequence
  k-mer
cgaacc

SEQ ID NO: 475 - DNA, 6 bp, Artificial Sequence
  k-mer
ggcgaa

SEQ ID NO: 476 - DNA, 6 bp, Artificial Sequence
  k-mer
gctcga

SEQ ID NO: 477 - DNA, 6 bp, Artificial Sequence
  k-mer
acgacc

SEQ ID NO: 478 - DNA, 6 bp, Artificial Sequence
  k-mer
cggtca

SEQ ID NO: 479 - DNA, 6 bp, Artificial Sequence
  k-mer
gcgata

SEQ ID NO: 480 - DNA, 6 bp, Artificial Sequence
  k-mer
cgcaac

SEQ ID NO: 481 - DNA, 6 bp, Artificial Sequence
  k-mer
cgaagc

SEQ ID NO: 482 - DNA, 6 bp, Artificial Sequence
  k-mer
gccgga

SEQ ID NO: 483 - DNA, 6 bp, Artificial Sequence
  k-mer
gcggaa

SEQ ID NO: 484 - DNA, 6 bp, Artificial Sequence
  k-mer
cgacaa

SEQ ID NO: 485 - DNA, 6 bp, Artificial Sequence
  k-mer
cttcgc

SEQ ID NO: 486 - DNA, 6 bp, Artificial Sequence
  k-mer
caaccg